European Patent Application EP 4 343 001 A1, published March 27, 2024. Title: METHOD FOR THE DIAGNOSIS OF ULCERATIVE COLITIS. Applicant: UNIVERSIDADE DE SANTIAGO DE COMPOSTELA. The sequence listing filed with the application follows.

SEQUENCE LISTING (18 sequences)

SEQ ID NO: 1 - DNA, 26 bp, synthetic construct
  source 1..26: mol_type = other DNA
  misc_feature 1..26: note = Target probe
tggcatcatgagttcacatgtccgca

SEQ ID NO: 2 - DNA, 113 bp, unidentified
  misc_feature 1..113: note = Amplification region
  source 1..113: mol_type = genomic DNA
gccagccttctgaaaggaagattaatccaggatggcatcatgagttcacatgtccgcagattaaaggtattttcggtagacgatggggatgcgttccattagatagtaggcgg

SEQ ID NO: 3 - DNA, 23 bp, synthetic construct
  misc_feature 1..23: note = REI forward primer
  source 1..23: mol_type = other DNA
cttggccagccttcttctgaaag

SEQ ID NO: 4 - DNA, 20 bp, synthetic construct
  source 1..20: mol_type = other DNA
  misc_feature 1..20: note = forward primer GENC4
gccagccttctgaaaggaag

SEQ ID NO: 5 - DNA, 22 bp, synthetic construct
  misc_feature 1..22: note = REI reverse primer
  source 1..22: mol_type = other DNA
ccccatcgtctaccgaaaatac

SEQ ID NO: 6 - DNA, 22 bp, synthetic construct
  source 1..22: mol_type = other DNA
ccgcctactatctaatggaacg

SEQ ID NO: 7 - DNA, 115 bp, Bacteroides dorei
  source 1..115: mol_type = genomic DNA
cttggccagccttctgaaaggaagattaatccaggatgggatcatgagttcacatgtccgcatgattaaaggtattttcggtagacgatggggatctactagtgcggccgcctgc

SEQ ID NO: 8 - DNA, 115 bp, Bacteroides vulgatus
  source 1..115: mol_type = genomic DNA
cttggccagccttctgaaaggaagattaatacaagatggcatcatgagtccgcatgttcacatgattaaaggtattttcggtagacgatggggatcccgcggccatggcggccgg

SEQ ID NO: 9 - DNA, 117 bp, unidentified
  misc_feature 1..117: note = Uncultured human fecal bacterium
  source 1..117: mol_type = genomic DNA
cttggccagccttctgaaaggaagattaatccaggatggcatcatgagttcacatgtccgcagattaaaggtattttcggtagacgatggggatgcgttccattagatagtaggcgg

SEQ ID NO: 10 - DNA, 115 bp, unidentified
  misc_feature 1..115: note = Uncultured human biopsy bacterium
  source 1..115: mol_type = genomic DNA
cttggccagccttctgaaaggaagattaatccaggatgggatcatgagttcacatgtccgcatgattaaaggtattttcggtatacgatggggatcccgcggccatggcggccgg

SEQ ID NO: 11 - DNA, 114 bp, unidentified
  misc_feature 1..114: note = Uncultured human biopsy bacterium
  source 1..114: mol_type = genomic DNA
cttggccagccttctgaaaggaagattaatccaggatggtatcatgagttcacatgtccgcatgattaaaggtattttcggtagacgatggggatctactagtgcggccgcctg

SEQ ID NO: 12 - DNA, 115 bp, unidentified
  misc_feature 1..115: note = Uncultured human biopsy bacterium
  source 1..115: mol_type = genomic DNA
cttggccagccttctgataggaagattaatccaggatgggatcatgagttcacatgtccgcatgattaaaggtattttcggtagacgatggggatcccgcggccatggcggccgg

SEQ ID NO: 13 - DNA, 115 bp, unidentified
  misc_feature 1..115: note = Uncultured human biopsy bacterium
  source 1..115: mol_type = genomic DNA
cttggccagccttctgaaatgaagattaatccaggatgggatcatgagttcacatgtccgcatgattaaaggtattttcggtagacgatggggatcccgcggccatggcggccgg

SEQ ID NO: 14 - DNA, 115 bp, unidentified
  misc_feature 1..115: note = Uncultured human biopsy bacterium
  source 1..115: mol_type = genomic DNA
cttggccagccttctgaaaggaagattaatgcaggatgggatcatgagttcacatgtccccatgagtaaaggtattttcggtagacgatggggatatagtagtgcggccgcctgc

SEQ ID NO: 15 - DNA, 114 bp, unidentified
  misc_feature 1..114: note = Uncultured human biopsy bacterium
  source 1..114: mol_type = genomic DNA
cttggccagccttctgaaaggaagattaatccaggatgggatcatgggttcacatgtccgcatgattaaggtattttcggtagacgatggggatcccgcggccatggcggccgg

SEQ ID NO: 16 - DNA, 20 bp, synthetic construct
  misc_feature 1..20: note = BacH forward primer
  source 1..20: mol_type = other DNA
cttggccagccttctgaaag

SEQ ID NO: 17 - DNA, 22 bp, synthetic construct
  misc_feature 1..22: note = BacH reverse primer
  source 1..22: mol_type = other DNA
ccccatcgtctaccgaaaatac

SEQ ID NO: 18 - DNA, 22 bp, unidentified
  source 1..22: mol_type = genomic DNA
cgttccattagatagtaggcgg